European Patent Application EP 4 378 958 A2, published June 5, 2024. Title: HIGH AFFINITY ANTI-MERTK ANTIBODIES AND USES THEREOF. Applicant: INSPIRNA, INC. The sequence listing filed with the application follows.

SEQUENCE LISTING (132 sequences)

SEQ ID NO: 1 - protein, 5 aa, synthetic construct
  source 1..5: note = Antibody z10/z11/z13/xAb VH CDR1 (Kabat)
NYGMN

SEQ ID NO: 2 - protein, 7 aa, synthetic construct
  source 1..7: note = Antibody z10/z11/z13/xAb VH CDR1 (Chothia)
GYTFTNY

SEQ ID NO: 3 - protein, 10 aa, synthetic construct
  source 1..10: note = Antibody z10/z11/z13/xAb VH CDR1 (AbM/Exemplary)
GYTFTNYGMN

SEQ ID NO: 4 - protein, 6 aa, synthetic construct
  source 1..6: note = Antibody z10/z11/z13/xAb VH CDR1 (Contact)
TNYGMN

SEQ ID NO: 5 - protein, 8 aa, synthetic construct
  source 1..8: note = Antibody z10/z11/z13/xAb VH CDR1 (IMGT)
GYTFTNYG

SEQ ID NO: 6 - protein, 17 aa, synthetic construct
  source 1..17: note = Antibody z10/z11/z13/xAb VH CDR2 (Kabat/Exemplary)
WINTYTGEPTYADDFKG

SEQ ID NO: 7 - protein, 4 aa, synthetic construct
  source 1..4: note = Antibody z10/z11/z13/xAb VH CDR2 (Chothia)
TYTG

SEQ ID NO: 8 - protein, 10 aa, synthetic construct
  source 1..10: note = Antibody z10/z11/z13/xAb VH CDR2 (AbM)
WINTYTGEPT

SEQ ID NO: 9 - protein, 13 aa, synthetic construct
  source 1..13: note = Antibody z10/z11/z13/xAb VH CDR2 (Contact)
WMGWINTYTGEPT

SEQ ID NO: 10 - protein, 8 aa, synthetic construct
  source 1..8: note = Antibody z10/z11/z13/xAb VH CDR2 (IMGT)
INTYTGEP

SEQ ID NO: 11 - protein, 11 aa, synthetic construct
  source 1..11: note = Antibody z10/z11/z13/xAb VH CDR3 (Kabat/AbM/Exemplary)
KSTVVSRYFDV

SEQ ID NO: 12 - protein, 9 aa, synthetic construct
  source 1..9: note = Antibody z10/z11/z13/xAb VH CDR3 (Chothia)
STVVSRYFD

SEQ ID NO: 13 - protein, 12 aa, synthetic construct
  source 1..12: note = Antibody z10/z11/z13/xAb VH CDR3 (Contact)
ARKSTVVSRYFD

SEQ ID NO: 14 - protein, 13 aa, synthetic construct
  source 1..13: note = Antibody z10/z11/z13/xAb VH CDR3 (IMGT)
ARKSTVVSRYFDV

SEQ ID NO: 15 - protein, 30 aa, synthetic construct
  source 1..30: note = Antibody z10/Z11/z13 VH Framework Region VH FR1 (Kabat)
QVQLVQSGAEVKKPGASVKVSCKASGYTFT

SEQ ID NO: 16 - protein, 14 aa, synthetic construct
  source 1..14: note = Antibody z10/z11/z13 VH Framework Region VH FR2 (Kabat)
WVRQAPGQGLEWMG

SEQ ID NO: 17 - protein, 32 aa, synthetic construct
  source 1..32: note = Antibody z10 VH Framework Region VH FR3 (Kabat/Exemplary)
RVTFTTDTSTSTAYMELRSLRSDDMAVYYCAR

SEQ ID NO: 18 - protein, 11 aa, synthetic construct
  source 1..11: note = Antibody z10/z11/z13 VH Framework Region VH FR4 (Kabat)
WGQGTTVTVSS

SEQ ID NO: 19 - protein, 25 aa, synthetic construct [sequence omitted]

SEQ ID NO: 20 - protein, 20 aa, synthetic construct
  source 1..20: note = Antibody z10/z11/z13 VH Framework Region VH FR2 (Chothia)
GMNWVRQAPGQGLEWMGWIN

SEQ ID NO: 21 - protein, 43 aa, synthetic construct
  source 1..43: note = Antibody z10 VH Framework Region VH FR3 (Chothia)
EPTYADDFKGRVTFTTDTSTSTAYMELRSLRSDDMAVYYCARK

SEQ ID NO: 22 - protein, 12 aa, synthetic construct
  source 1..12: note = Antibody z10/z11/z13 VH Framework Region VH FR4 (Chothia)
VWGQGTTVTVSS

SEQ ID NO: 23 - protein, 25 aa, synthetic construct [sequence omitted]

SEQ ID NO: 24 - protein, 14 aa, synthetic construct
  source 1..14: note = Antibody z10/z11/z13 VH Framework Region VH FR2 (AbM)
WVRQAPGQGLEWMG

SEQ ID NO: 25 - protein, 39 aa, synthetic construct
  source 1..39: note = Antibody z10 VH Framework Region VH FR3 (AbM)
YADDFKGRVTFTTDTSTSTAYMELRSLRSDDMAVYYCAR

SEQ ID NO: 26 - protein, 11 aa, synthetic construct
  source 1..11: note = Antibody z10/z11/z13 VH Framework Region VH FR4 (AbM)
WGQGTTVTVSS

SEQ ID NO: 27 - protein, 29 aa, synthetic construct
  source 1..29: note = Antibody z10/z11/z13 VH Framework Region VH FR1 (Contact)
QVQLVQSGAEVKKPGASVKVSCKASGYTF

SEQ ID NO: 28 - protein, 11 aa, synthetic construct
  source 1..11: note = Antibody z10/z11/z13 VH Framework Region VH FR2 (Contact)
WVRQAPGQGLE

SEQ ID NO: 29 - protein, 37 aa, synthetic construct
  source 1..37: note = Antibody z10 VH Framework Region VH FR3 (Contact)
YADDFKGRVTFTTDTSTSTAYMELRSLRSDDMAVYYC

SEQ ID NO: 30 - protein, 12 aa, synthetic construct
  source 1..12: note = Antibody z10/z11/z13 VH Framework Region VH FR4 (Contact)
VWGQGTTVTVSS

SEQ ID NO: 31 - protein, 25 aa, synthetic construct [sequence omitted]

SEQ ID NO: 32 - protein, 17 aa, synthetic construct
  source 1..17: note = Antibody z10/z11/z13 VH Framework Region VH FR2 (IMGT)
MNWVRQAPGQGLEWMGW

SEQ ID NO: 33 - protein, 38 aa, synthetic construct
  source 1..38: note = Antibody z10 VH Framework Region VH FR3 (IMGT)
TYADDFKGRVTFTTDTSTSTAYMELRSLRSDDMAVYYC

SEQ ID NO: 34 - protein, 11 aa, synthetic construct
  source 1..11: note = Antibody z10/z11/z13 VH Framework Region VH FR4 (IMGT)
WGQGTTVTVSS

SEQ ID NO: 35 - protein, 25 aa, synthetic construct [sequence omitted]

SEQ ID NO: 36 - protein, 14 aa, synthetic construct
  source 1..14: note = Antibody z10/z11/z13 VH Framework Region VH FR2 (Exemplary)
WVRQAPGQGLEWMG

SEQ ID NO: 37 - protein, 11 aa, synthetic construct
  source 1..11: note = Antibody z10/z11/z13 VH Framework Region VH FR4 (Exemplary)
WGQGTTVTVSS

SEQ ID NO: 38 - protein, 32 aa, synthetic construct
  source 1..32: note = Antibody z11 VH Framework Region VH FR3 (Kabat/Exemplary)
RVTMTLDTSTSTAYMELRSLRSDDMAVYYCAR

SEQ ID NO: 39 - protein, 43 aa, synthetic construct
  source 1..43: note = Antibody z11 VH Framework Region VH FR3 (Chothia)
EPTYADDFKGRVTMTLDTSTSTAYMELRSLRSDDMAVYYCARK

SEQ ID NO: 40 - protein, 39 aa, synthetic construct
  source 1..39: note = Antibody z11 VH Framework Region VH FR3 (AbM)
YADDFKGRVTMTLDTSTSTAYMELRSLRSDDMAVYYCAR

SEQ ID NO: 41 - protein, 37 aa, synthetic construct
  source 1..37: note = Antibody z11 VH Framework Region VH FR3 (Contact)
YADDFKGRVTMTLDTSTSTAYMELRSLRSDDMAVYYC

SEQ ID NO: 42 - protein, 38 aa, synthetic construct
  source 1..38: note = Antibody z11 VH Framework Region VH FR3 (IMGT)
TYADDFKGRVTMTLDTSTSTAYMELRSLRSDDMAVYYC

SEQ ID NO: 43 - protein, 32 aa, synthetic construct
  source 1..32: note = Antibody z13 VH Framework Region VH FR3 (Kabat/Exemplary)
RVTFTLDTSTSTAYMELRSLRSDDMAVYYCAR

SEQ ID NO: 44 - protein, 43 aa, synthetic construct
  source 1..43: note = Antibody z13 VH Framework Region VH FR3 (Chothia)
EPTYADDFKGRVTFTLDTSTSTAYMELRSLRSDDMAVYYCARK

SEQ ID NO: 45 - protein, 39 aa, synthetic construct
  source 1..39: note = Antibody z13 VH Framework Region VH FR3 (AbM)
YADDFKGRVTFTLDTSTSTAYMELRSLRSDDMAVYYCAR

SEQ ID NO: 46 - protein, 37 aa, synthetic construct
  source 1..37: note = Antibody z13 VH Framework Region VH FR3 (Contact)
YADDFKGRVTFTLDTSTSTAYMELRSLRSDDMAVYYC

SEQ ID NO: 47 - protein, 38 aa, synthetic construct
  source 1..38: note = Antibody z13 VH Framework Region VH FR3 (IMGT)
TYADDFKGRVTFTLDTSTSTAYMELRSLRSDDMAVYYC

SEQ ID NO: 48 - protein, 32 aa, synthetic construct
  VARIANT 4: note = misc_feature - Xaa = Phe or Met
  VARIANT 6: note = misc_feature - Xaa = Thr or Leu
  source 1..32: note = Antibody VH FR3 Consensus sequence (Kabat)
RVTXTXDTSTSTAYMELRSLRSDDMAVYYCAR

SEQ ID NO: 49 - protein, 43 aa, synthetic construct
  VARIANT 14: note = misc_feature - Xaa = Phe or Met
  VARIANT 16: note = misc_feature - Xaa = Thr or Leu
  source 1..43: note = Antibody VH FR3 Consensus sequence (Chothia)
EPTYADDFKGRVTXTXDTSTSTAYMELRSLRSDDMAVYYCARK

SEQ ID NO: 50 - protein, 39 aa, synthetic construct
  VARIANT 11: note = misc_feature - Xaa = Phe or Met
  VARIANT 13: note = misc_feature - Xaa = Thr or Leu
  source 1..39: note = Antibody VH FR3 Consensus sequence (AbM)
YADDFKGRVTXTXDTSTSTAYMELRSLRSDDMAVYYCAR

SEQ ID NO: 51 - protein, 37 aa, synthetic construct
  VARIANT 11: note = misc_feature - Xaa = Phe or Met
  VARIANT 13: note = misc_feature - Xaa = Thr or Leu
  source 1..37: note = Antibody VH FR3 Consensus sequence (Contact)
YADDFKGRVTXTXDTSTSTAYMELRSLRSDDMAVYYC

SEQ ID NO: 52 - protein, 38 aa, synthetic construct
  VARIANT 12: note = misc_feature - Xaa = Phe or Met
  VARIANT 14: note = misc_feature - Xaa = Thr or Leu
  source 1..38: note = Antibody VH FR3 Consensus sequence (IMGT)
TYADDFKGRVTXTXDTSTSTAYMELRSLRSDDMAVYYC

SEQ ID NO: 53 - protein, 32 aa, synthetic construct; identical to SEQ ID NO: 48
  VARIANT 4: note = misc_feature - Xaa = Phe or Met
  VARIANT 6: note = misc_feature - Xaa = Thr or Leu
  source 1..32: note = Antibody VH FR3 Consensus sequence (Exemplary)

SEQ ID NO: 54 - protein, 30 aa, synthetic construct
  source 1..30: note = Antibody xAb VH Framework Region VH FR1 (Kabat)
QIQLVQSGPELKKPGETVKISCKASGYTFT

SEQ ID NO: 55 - protein, 14 aa, synthetic construct
  source 1..14: note = Antibody xAb VH Framework Region VH FR2 (Kabat/AbM/Exemplary)
WVKQAPGKGLKWMG

SEQ ID NO: 56 - protein, 32 aa, synthetic construct
  source 1..32: note = Antibody xAb VH Framework Region VH FR3 (Kabat/Exemplary)
RFVFSLETSASTAYLQINNLKNEDMATYFCAR

SEQ ID NO: 57 - protein, 11 aa, synthetic construct
  source 1..11: note = Antibody xAb VH Framework Region VH FR4 (Kabat/AbM/IMGT/Exemplary)
WGAGTTVTVSS

SEQ ID NO: 58 - protein, 25 aa, synthetic construct
  source 1..25: note = Antibody xAb VH Framework Region VH FR1 (Chothia/AbM/IMGT/Exemplary)
QIQLVQSGPELKKPGETVKISCKAS

SEQ ID NO: 59 - protein, 20 aa, synthetic construct
  source 1..20: note = Antibody xAb VH Framework Region VH FR2 (Chothia)
GMNWVKQAPGKGLKWMGWIN

SEQ ID NO: 60 - protein, 43 aa, synthetic construct
  source 1..43: note = Antibody xAb VH Framework Region VH FR3 (Chothia)
EPTYADDFKGRFVFSLETSASTAYLQINNLKNEDMATYFCARK

SEQ ID NO: 61 - protein, 12 aa, synthetic construct
  source 1..12: note = Antibody xAb VH Framework Region VH FR4 (Chothia/Contact)
VWGAGTTVTVSS

SEQ ID NO: 62 - protein, 39 aa, synthetic construct
  source 1..39: note = Antibody xAb VH Framework Region VH FR3 (AbM)
YADDFKGRFVFSLETSASTAYLQINNLKNEDMATYFCAR

SEQ ID NO: 63 - protein, 29 aa, synthetic construct
  source 1..29: note = Antibody xAb VH Framework Region VH FR1 (Contact)
QIQLVQSGPELKKPGETVKISCKASGYTF

SEQ ID NO: 64 - protein, 11 aa, synthetic construct
  source 1..11: note = Antibody xAb VH Framework Region VH FR2 (Contact)
WVKQAPGKGLK

SEQ ID NO: 65 - protein, 37 aa, synthetic construct
  source 1..37: note = Antibody xAb VH Framework Region VH FR3 (Contact)
YADDFKGRFVFSLETSASTAYLQINNLKNEDMATYFC

SEQ ID NO: 66 - protein, 17 aa, synthetic construct
  source 1..17: note = Antibody xAb VH Framework Region VH FR2 (IMGT)
MNWVKQAPGKGLKWMGW

SEQ ID NO: 67 - protein, 38 aa, synthetic construct
  source 1..38: note = Antibody xAb VH Framework Region VH FR3 (IMGT)
TYADDFKGRFVFSLETSASTAYLQINNLKNEDMATYFC

SEQ ID NO: 68 - protein, 11 aa, synthetic construct
  source 1..11: note = Antibody z10/z11/z13/xAb VL CDR1 (Kabat/AbM/Exemplary)
KASQDVGDAVT

SEQ ID NO: 69 - protein, 7 aa, synthetic construct
  source 1..7: note = Antibody z10/z11/z13/xAb VL CDR2 (Kabat/AbM/Exemplary)
WASTRHT

SEQ ID NO: 70 - protein, 9 aa, synthetic construct
  source 1..9: note = Antibody z10/z11/z13/xAb VL CDR3 (Kabat/AbM/IMGT/Exemplary)
QQYRSYPLT

SEQ ID NO: 71 - protein, 7 aa, synthetic construct
  source 1..7: note = Antibody z10/z11/z13/xAb VL CDR1 (Chothia)
SQDVGDA

SEQ ID NO: 72 - skipped

SEQ ID NO: 73 - protein, 6 aa, synthetic construct
  source 1..6: note = Antibody z10/z11/z13/xAb VL CDR3 (Chothia)
YRSYPL

SEQ ID NO: 74 - protein, 7 aa, synthetic construct
  source 1..7: note = Antibody z10/z11/z13 VL CDR1 (Contact)
GDAVTWY

SEQ ID NO: 75 - protein, 10 aa, synthetic construct
  source 1..10: note = Antibody z10/z11/z13/xAb VL CDR2 (Contact)
LLIYWASTRH

SEQ ID NO: 76 - protein, 8 aa, synthetic construct
  source 1..8: note = Antibody z10/z11/z13/xAb VL CDR3 (Contact)
QQYRSYPL

SEQ ID NO: 77 - protein, 6 aa, synthetic construct
  source 1..6: note = Antibody z10/z11/z13/xAb VL CDR1 (IMGT)
QDVGDA

SEQ ID NO: 78 - protein, 7 aa, synthetic construct
  source 1..7: note = Antibody xAb VL CDR1 (Contact)
GDAVTWC

SEQ ID NO: 79 - protein, 23 aa, synthetic construct
  source 1..23: note = Antibody z10/z11/z13 VL Framework Region VL FR1 (Kabat/AbM/Exemplary)
DIQMTQSPSFLSASVGDRVTITC

SEQ ID NO: 80 - protein, 15 aa, synthetic construct
  source 1..15: note = Antibody z10/z11/z13 VL Framework Region VL FR2 (Kabat/AbM/Exemplary)
WYQQKPGKAPKLLIY

SEQ ID NO: 81 - protein, 32 aa, synthetic construct
  source 1..32: note = Antibody z10/z11/z13 VL Framework Region VL FR3 (Kabat/AbM/Exemplary)
GVPDRFSGSGSGTDFTLTISSLQPEDFATYYC

SEQ ID NO: 82 - protein, 10 aa, synthetic construct
  source 1..10: note = Antibody z10/z11/z13 VL Framework Region VL FR4 (Kabat/AbM/IMGT/Exemplary)
FGQGTKLEIK

SEQ ID NO: 83 - protein, 25 aa, synthetic construct
  source 1..25: note = Antibody z10/z11/z13 VL Framework Region VL FR1 (Chothia)
DIQMTQSPSFLSASVGDRVTITCKA

SEQ ID NO: 84 - protein, 17 aa, synthetic construct
  source 1..17: note = Antibody z10/z11/z13 VL Framework Region VL FR2 (Chothia/IMGT)
VTWYQQKPGKAPKLLIY

SEQ ID NO: 85 - protein, 38 aa, synthetic construct
  source 1..38: note = Antibody z10/z11/z13 VL Framework Region VL FR3 (Chothia)
TRHTGVPDRFSGSGSGTDFTLTISSLQPEDFATYYCQQ

SEQ ID NO: 86 - protein, 11 aa, synthetic construct
  source 1..11: note = Antibody z10/z11/z13 VL Framework Region VL FR4 (Chothia/Contact)
TFGQGTKLEIK

SEQ ID NO: 87 - protein, 29 aa, synthetic construct
  source 1..29: note = Antibody z10/z11/z13 VL Framework Region VL FR1 (Contact)
DIQMTQSPSFLSASVGDRVTITCKASQDV

SEQ ID NO: 88 - protein, 9 aa, synthetic construct
  source 1..9: note = Antibody z10/z11/z13 VL Framework Region VL FR2 (Contact)
QQKPGKAPK

SEQ ID NO: 89 - protein, 33 aa, synthetic construct
  source 1..33: note = Antibody z10/z11/z13 VL Framework Region VL FR3 (Contact)
TGVPDRFSGSGSGTDFTLTISSLQPEDFATYYC

SEQ ID NO: 90 - protein, 26 aa, synthetic construct
  source 1..26: note = Antibody z10/z11/z13 VL Framework Region VL FR1 (IMGT)
DIQMTQSPSFLSASVGDRVTITCKAS

SEQ ID NO: 91 - protein, 36 aa, synthetic construct
  source 1..36: note = Antibody z10/z11/z13 VL Framework Region VL FR3 (IMGT)
TRHTGVPDRFSGSGSGTDFTLTISSLQPEDFATYYC

SEQ ID NO: 92 - protein, 23 aa, synthetic construct
  source 1..23: note = Antibody xAb VL Framework Region VL FR1 (Kabat/AbM/Exemplary)
DIVLTQSHKFMSTSVGDRVSITC

SEQ ID NO: 93 - protein, 15 aa, synthetic construct
  source 1..15: note = Antibody xAb VL Framework Region VL FR2 (Kabat/AbM/Exemplary)
WCQQKPGQPPKLLIY

SEQ ID NO: 94 - protein, 32 aa, synthetic construct
  source 1..32: note = Antibody xAb VL Framework Region VL FR3 (Kabat/AbM/Exemplary)
GVPDRFTGSGSGTDFTLTINNVQSEDLADYFC

SEQ ID NO: 95 - protein, 10 aa, synthetic construct
  source 1..10: note = Antibody xAb VL Framework Region VL FR4 (Kabat/AbM/IMGT/Exemplary)
FGAGTKLELK

SEQ ID NO: 96 - protein, 25 aa, synthetic construct
  source 1..25: note = Antibody xAb VL Framework Region VL FR1 (Chothia)
DIVLTQSHKFMSTSVGDRVSITCKA

SEQ ID NO: 97 - protein, 17 aa, synthetic construct
  source 1..17: note = Antibody xAb VL Framework Region VL FR2 (Chothia/IMGT)
VTWCQQKPGQPPKLLIY

SEQ ID NO: 98 - protein, 38 aa, synthetic construct
  source 1..38: note = Antibody xAb VL Framework Region VL FR3 (Chothia)
TRHTGVPDRFTGSGSGTDFTLTINNVQSEDLADYFCQQ

SEQ ID NO: 99 - protein, 11 aa, synthetic construct
  source 1..11: note = Antibody xAb VL Framework Region VL FR4 (Chothia/Contact)
TFGAGTKLELK

SEQ ID NO: 100 - protein, 29 aa, synthetic construct
  source 1..29: note = Antibody xAb VL Framework Region VL FR1 (Contact)
DIVLTQSHKFMSTSVGDRVSITCKASQDV

SEQ ID NO: 101 - protein, 9 aa, synthetic construct
  source 1..9: note = Antibody xAb VL Framework Region VL FR2 (Contact)
QQKPGQPPK

SEQ ID NO: 102 - protein, 33 aa, synthetic construct
  source 1..33: note = Antibody xAb VL Framework Region VL FR3 (Contact)
TGVPDRFTGSGSGTDFTLTINNVQSEDLADYFC

SEQ ID NO: 103 - protein, 26 aa, synthetic construct
  source 1..26: note = Antibody xAb VL Framework Region VL FR1 (IMGT)
DIVLTQSHKFMSTSVGDRVSITCKAS

SEQ ID NO: 104 - protein, 36 aa, synthetic construct
  source 1..36: note = Antibody xAb VL Framework Region VL FR3 (IMGT)
TRHTGVPDRFTGSGSGTDFTLTINNVQSEDLADYFC

SEQ ID NO: 105 - protein, 120 aa, synthetic construct
  source 1..120: note = Antibody z10 Heavy Chain Variable Region (VH)
QVQLVQSGAEVKKPGASVKVSCKASGYTFTNYGMNWVRQAPGQGLEWMGWINTYTGEPTYADDFKGRVTFTTDTSTSTAYMELRSLRSDDMAVYYCARKSTVVSRYFDVWGQGTTVTVSS

SEQ ID NO: 106 - protein, 107 aa, synthetic construct
  source 1..107: note = Antibody z10/z11/z13 light Chain Variable Region (VL)
DIQMTQSPSFLSASVGDRVTITCKASQDVGDAVTWYQQKPGKAPKLLIYWASTRHTGVPDRFSGSGSGTDFTLTISSLQPEDFATYYCQQYRSYPLTFGQGTKLEIK

SEQ ID NO: 107 - protein, 120 aa, synthetic construct
  source 1..120: note = Antibody z11 Heavy Chain Variable Region (VH)
QVQLVQSGAEVKKPGASVKVSCKASGYTFTNYGMNWVRQAPGQGLEWMGWINTYTGEPTYADDFKGRVTMTLDTSTSTAYMELRSLRSDDMAVYYCARKSTVVSRYFDVWGQGTTVTVSS

SEQ ID NO: 108 - protein, 120 aa, synthetic construct
  source 1..120: note = Antibody z13 Heavy Chain Variable Region (VH)
QVQLVQSGAEVKKPGASVKVSCKASGYTFTNYGMNWVRQAPGQGLEWMGWINTYTGEPTYADDFKGRVTFTLDTSTSTAYMELRSLRSDDMAVYYCARKSTVVSRYFDVWGQGTTVTVSS

SEQ ID NO: 109 - protein, 120 aa, synthetic construct
  VARIANT 70: note = misc_feature - Xaa = Phe or Met
  VARIANT 72: note = misc_feature - Xaa = Thr or Leu
  source 1..120: note = Antibody Heavy Chain Variable Region Consensus sequence
QVQLVQSGAEVKKPGASVKVSCKASGYTFTNYGMNWVRQAPGQGLEWMGWINTYTGEPTYADDFKGRVTXTXDTSTSTAYMELRSLRSDDMAVYYCARKSTVVSRYFDVWGQGTTVTVSS

SEQ ID NO: 110 - protein, 120 aa, synthetic construct
  source 1..120: note = Antibody xAb Heavy Chain Variable Region (VH)
QIQLVQSGPELKKPGETVKISCKASGYTFTNYGMNWVKQAPGKGLKWMGWINTYTGEPTYADDFKGRFVFSLETSASTAYLQINNLKNEDMATYFCARKSTVVSRYFDVWGAGTTVTVSS

SEQ ID NO: 111 - protein, 107 aa, synthetic construct
  source 1..107: note = Antibody xAb Light Chain Variable Region (VL)
DIVLTQSHKFMSTSVGDRVSITCKASQDVGDAVTWCQQKPGQPPKLLIYWASTRHTGVPDRFTGSGSGTDFTLTINNVQSEDLADYFCQQYRSYPLTFGAGTKLELK

SEQ ID NO: 112 - protein, 450 aa, synthetic construct
  source 1..450: note = Antibody z10 Heavy Chain
QVQLVQSGAEVKKPGASVKVSCKASGYTFTNYGMNWVRQAPGQGLEWMGWINTYTGEPTYADDFKGRVTFTTDTSTSTAYMELRSLRSDDMAVYYCARKSTVVSRYFDVWGQGTTVTVSSASTKGPSVFPLAPSSKSTSGGTAALGCLVKDYFPEPVTVSWNSGALTSGVHTFPAVLQSSGLYSLSSVVTVPSSSLGTQTYICNVNHKPSNTKVDKRVEPKSCDKTHTCPPCPAPELLGGPSVFLFPPKPKDTLMISRTPEVTCVVVDVSHEDPEVKFNWYVDGVEVHNAKTKPREEQYNSTYRVVSVLTVLHQDWLNGKEYKCKVSNKALPAPIEKTISKAKGQPREPQVYTLPPSREEMTKNQVSLTCLVKGFYPSDIAVEWESNGQPENNYKTTPPVLDSDGSFFLYSKLTVDKSRWQQGNVFSCSVMHEALHNHYTQKSLSLSPGK

SEQ ID NO: 113 - protein, 214 aa, synthetic construct
  source 1..214: note = Antibody z10/z11/z13 Light Chain
DIQMTQSPSFLSASVGDRVTITCKASQDVGDAVTWYQQKPGKAPKLLIYWASTRHTGVPDRFSGSGSGTDFTLTISSLQPEDFATYYCQQYRSYPLTFGQGTKLEIKRTVAAPSVFIFPPSDEQLKSGTASVVCLLNNFYPREAKVQWKVDNALQSGNSQESVTEQDSKDSTYSLSSTLTLSKADYEKHKVYACEVTHQGLSSPVTKSFNRGEC

SEQ ID NO: 114 - protein, 450 aa, synthetic construct
  source 1..450: note = Antibody z11 Heavy Chain
QVQLVQSGAEVKKPGASVKVSCKASGYTFTNYGMNWVRQAPGQGLEWMGWINTYTGEPTYADDFKGRVTMTLDTSTSTAYMELRSLRSDDMAVYYCARKSTVVSRYFDVWGQGTTVTVSSASTKGPSVFPLAPSSKSTSGGTAALGCLVKDYFPEPVTVSWNSGALTSGVHTFPAVLQSSGLYSLSSVVTVPSSSLGTQTYICNVNHKPSNTKVDKRVEPKSCDKTHTCPPCPAPELLGGPSVFLFPPKPKDTLMISRTPEVTCVVVDVSHEDPEVKFNWYVDGVEVHNAKTKPREEQYNSTYRVVSVLTVLHQDWLNGKEYKCKVSNKALPAPIEKTISKAKGQPREPQVYTLPPSREEMTKNQVSLTCLVKGFYPSDIAVEWESNGQPENNYKTTPPVLDSDGSFFLYSKLTVDKSRWQQGNVFSCSVMHEALHNHYTQKSLSLSPGK

SEQ ID NO: 115 - protein, 450 aa, synthetic construct
  source 1..450: note = Antibody z13 Heavy Chain
QVQLVQSGAEVKKPGASVKVSCKASGYTFTNYGMNWVRQAPGQGLEWMGWINTYTGEPTYADDFKGRVTFTLDTSTSTAYMELRSLRSDDMAVYYCARKSTVVSRYFDVWGQGTTVTVSSASTKGPSVFPLAPSSKSTSGGTAALGCLVKDYFPEPVTVSWNSGALTSGVHTFPAVLQSSGLYSLSSVVTVPSSSLGTQTYICNVNHKPSNTKVDKRVEPKSCDKTHTCPPCPAPELLGGPSVFLFPPKPKDTLMISRTPEVTCVVVDVSHEDPEVKFNWYVDGVEVHNAKTKPREEQYNSTYRVVSVLTVLHQDWLNGKEYKCKVSNKALPAPIEKTISKAKGQPREPQVYTLPPSREEMTKNQVSLTCLVKGFYPSDIAVEWESNGQPENNYKTTPPVLDSDGSFFLYSKLTVDKSRWQQGNVFSCSVMHEALHNHYTQKSLSLSPGK

SEQ ID NO: 116 - protein, 450 aa, synthetic construct
  VARIANT 70: note = misc_feature - Xaa = Phe or Met
  VARIANT 72: note = misc_feature - Xaa = Thr or Leu
  source 1..450: note = Antibody Heavy Chain Consensus Sequences
QVQLVQSGAEVKKPGASVKVSCKASGYTFTNYGMNWVRQAPGQGLEWMGWINTYTGEPTYADDFKGRVTXTXDTSTSTAYMELRSLRSDDMAVYYCARKSTVVSRYFDVWGQGTTVTVSSASTKGPSVFPLAPSSKSTSGGTAALGCLVKDYFPEPVTVSWNSGALTSGVHTFPAVLQSSGLYSLSSVVTVPSSSLGTQTYICNVNHKPSNTKVDKRVEPKSCDKTHTCPPCPAPELLGGPSVFLFPPKPKDTLMISRTPEVTCVVVDVSHEDPEVKFNWYVDGVEVHNAKTKPREEQYNSTYRVVSVLTVLHQDWLNGKEYKCKVSNKALPAPIEKTISKAKGQPREPQVYTLPPSREEMTKNQVSLTCLVKGFYPSDIAVEWESNGQPENNYKTTPPVLDSDGSFFLYSKLTVDKSRWQQGNVFSCSVMHEALHNHYTQKSLSLSPGK

SEQ ID NO: 117 - protein, 450 aa, synthetic construct
  source 1..450: note = Antibody xAb Heavy Chain
QIQLVQSGPELKKPGETVKISCKASGYTFTNYGMNWVKQAPGKGLKWMGWINTYTGEPTYADDFKGRFVFSLETSASTAYLQINNLKNEDMATYFCARKSTVVSRYFDVWGAGTTVTVSSASTKGPSVFPLAPSSKSTSGGTAALGCLVKDYFPEPVTVSWNSGALTSGVHTFPAVLQSSGLYSLSSVVTVPSSSLGTQTYICNVNHKPSNTKVDKRVEPKSCDKTHTCPPCPAPELLGGPSVFLFPPKPKDTLMISRTPEVTCVVVDVSHEDPEVKFNWYVDGVEVHNAKTKPREEQYNSTYRVVSVLTVLHQDWLNGKEYKCKVSNKALPAPIEKTISKAKGQPREPQVYTLPPSREEMTKNQVSLTCLVKGFYPSDIAVEWESNGQPENNYKTTPPVLDSDGSFFLYSKLTVDKSRWQQGNVFSCSVMHEALHNHYTQKSLSLSPGK

SEQ ID NO: 118 - protein, 214 aa, synthetic construct
  source 1..214: note = Antibody xAb Light Chain
DIVLTQSHKFMSTSVGDRVSITCKASQDVGDAVTWCQQKPGQPPKLLIYWASTRHTGVPDRFTGSGSGTDFTLTINNVQSEDLADYFCQQYRSYPLTFGAGTKLELKRTVAAPSVFIFPPSDEQLKSGTASVVCLLNNFYPREAKVQWKVDNALQSGNSQESVTEQDSKDSTYSLSSTLTLSKADYEKHKVYACEVTHQGLSSPVTKSFNRGEC

SEQ ID NO: 119 - DNA, 360 bp, synthetic construct
  source 1..360: mol_type = other DNA; note = Antibody z10 Variable Region VH DNA Sequences
caggtgcagctggtgcagagcggcgctgaggtgaagaagcccggcgctagcgtgaaggtgagctgcaaggccagcggctacaccttcaccaactacggcatgaactgggtgaggcaggctcctggacagggcctggagtggatgggctggatcaacacatacaccggcgagcccacctacgccgacgacttcaagggcagggtgacctttaccaccgacaccagcaccagcaccgcctacatggagctgaggagcctgagaagcgacgacatggccgtgtactactgcgccagaaagagcaccgtggtgtccaggtacttcgacgtgtggggccagggcaccacagtgaccgtgagcagc

SEQ ID NO: 120 - DNA, 321 bp, synthetic construct
  source 1..321: mol_type = other DNA; note = Antibody z10/z11/z13 Variable Region VL DNA Sequences
gacatccagatgacccagagccccagcttcctgtccgctagcgtgggcgacagggtgaccatcacctgcaaggccagccaggacgtgggcgatgccgtgacctggtatcagcagaagcccggcaaggcccccaagctgctgatctactgggccagcacaaggcacacaggcgtgcccgacagattcagcggcagcggaagcggcaccgacttcaccctgaccatcagcagcctgcagcccgaggacttcgccacctactactgccagcagtacaggagctaccccctgaccttcggccagggcaccaagctggaaatcaag

SEQ ID NO: 121 - DNA, 360 bp, synthetic construct
  source 1..360: mol_type = other DNA; note = Antibody z11 Variable Region VH DNA Sequences
caggtgcagctggtgcagagcggagccgaggtgaagaagcctggcgccagcgtgaaggtgagctgcaaggccagcggctacaccttcaccaactacggcatgaactgggtgaggcaggctcctggccagggactggagtggatgggctggatcaacacctacaccggcgagcccacctacgccgacgacttcaagggcagggtgaccatgaccctggacaccagcaccagcaccgcctacatggagctgaggagcctgaggagcgacgacatggccgtgtactactgcgccaggaagagcaccgtggtgtccaggtacttcgacgtgtggggacagggcaccaccgtgaccgtgagcagc

SEQ ID NO: 122 - DNA, 360 bp, synthetic construct
  source 1..360: mol_type = other DNA; note = Antibody z13 Variable Region VH DNA Sequences
caggtgcagctggtgcagagcggagccgaagtgaagaagcccggcgccagcgtgaaggtgagctgcaaggccagcggctacaccttcaccaactacggcatgaactgggtgagacaggcccctggacagggactggagtggatgggctggatcaacacctacaccggcgagcccacctacgccgacgacttcaagggcagggtgaccttcaccctggacaccagcaccagcaccgcctacatggagctgaggagcctgaggagcgacgacatggccgtgtactattgcgccaggaagagcaccgtggtgagcaggtacttcgacgtgtggggccagggaaccaccgtgaccgtgagcagc

SEQ ID NO: 123 - DNA, 360 bp, synthetic construct
  source 1..360: mol_type = other DNA; note = Antibody xAb Variable Region VH DNA Sequences
cagatccagttggtgcagtctggacctgagctgaagaagcctggagagacagtcaagatctcctgcaaggcttctggatataccttcacaaactatggaatgaactgggtgaagcaggctccaggaaagggtttaaagtggatgggctggataaacacctacactggagagccaacatatgctgatgacttcaagggacggtttgtcttctctttggaaacctctgccagcactgcctacttgcagatcaacaacctcaaaaatgaggacatggccacatatttctgtgcaagaaaaagtacggtagtaagtaggtacttcgatgtctggggcgcagggaccacggtcaccgtctcctca

SEQ ID NO: 124 - DNA, 321 bp, synthetic construct
  source 1..321: mol_type = other DNA; note = Antibody xAb Variable Region VL DNA Sequences
gacattgtgctgacccagtctcacaaattcatgtccacatcagtaggagacagggtcagcatcacctgcaaggccagtcaggatgtgggtgatgctgtaacctggtgtcaacagaaaccaggtcaacctcctaaactactgatttactgggcatccacccggcacactggagtccctgatcgcttcacaggcagtgggtctgggacagatttcactctcaccattaacaatgtgcagtctgaggacttggcagattatttctgtcagcaatatcgcagctatcctctcacgttcggtgctgggaccaagctggagctgaaa

SEQ ID NO: 125 - DNA, 1353 bp, synthetic construct
  source 1..1353: mol_type = other DNA; note = Antibody z10 Heavy Chain DNA Sequences
caggtgcagctggtgcagagcggcgctgaggtgaagaagcccggcgctagcgtgaaggtgagctgcaaggccagcggctacaccttcaccaactacggcatgaactgggtgaggcaggctcctggacagggcctggagtggatgggctggatcaacacatacaccggcgagcccacctacgccgacgacttcaagggcagggtgacctttaccaccgacaccagcaccagcaccgcctacatggagctgaggagcctgagaagcgacgacatggccgtgtactactgcgccagaaagagcaccgtggtgtccaggtacttcgacgtgtggggccagggcaccacagtgaccgtgagcagcgcgtcgaccaagggcccatccgtcttccccctggcaccctcctccaagagcacctctgggggcacagcggccctgggctgcctggtcaaggactacttccccgaaccggtgacggtgtcctggaactcaggcgctctgaccagcggcgtgcacaccttcccggctgtcctacagtcctcaggactctactccctcagcagcgtggtgaccgtgccctccagcagcttgggcacccagacctacatctgcaacgtgaatcacaagcccagcaacaccaaggtggacaagagagttgagcccaaatcttgtgacaaaactcacacatgcccaccgtgcccagcacctgaactcctggggggaccgtcagtcttcctcttccccccaaaacccaaggacaccctcatgatctcccggacccctgaggtcacatgcgtggtggtggacgtgagccacgaagaccctgaggtcaagttcaactggtacgtggacggcgtggaggtgcataatgccaagacaaagccgcgggaggagcagtacaacagcacgtaccgtgtggtcagcgtcctcaccgtcctgcaccaggactggctgaatggcaaggagtacaagtgcaaggtctccaacaaagccctcccagcccccatcgagaaaaccatctccaaagccaaagggcagccccgagaaccacaggtctacaccctgcccccatcccgggaggagatgaccaagaaccaggtcagcctgacctgcctggtcaaaggcttctatcccagcgacatcgccgtggagtgggagagcaatgggcagccggagaacaactacaagaccacgcctcccgtgctggactccgacggctccttcttcctctatagcaagctcaccgtggacaagagcaggtggcagcaggggaacgtcttctcatgctccgtgatgcatgaggctctgcacaaccactacacgcagaagagcttaagcctgtctccgggtaaatga

SEQ ID NO: 126 - DNA, 645 bp, synthetic construct
  source 1..645: mol_type = other DNA; note = Antibody z10/z11/z13 Light Chain DNA Sequences
gacatccagatgacccagagccccagcttcctgtccgctagcgtgggcgacagggtgaccatcacctgcaaggccagccaggacgtgggcgatgccgtgacctggtatcagcagaagcccggcaaggcccccaagctgctgatctactgggccagcacaaggcacacaggcgtgcccgacagattcagcggcagcggaagcggcaccgacttcaccctgaccatcagcagcctgcagcccgaggacttcgccacctactactgccagcagtacaggagctaccccctgaccttcggccagggcaccaagctggaaatcaagcgtacggtggctgcaccatctgtcttcatcttcccgccatctgatgagcagttgaaatctggaactgcctctgttgtgtgcctgctgaataacttctatcccagagaggccaaagtacagtggaaggtggataacgccctccaatcgggtaactcccaggagagtgtcacagagcaggacagcaaggacagcacctacagcctcagcagcaccctgacgctgagcaaagcagactacgagaaacacaaagtctacgcctgcgaagtcacccatcagggcctgagctcgcccgtcacaaagagcttcaacaggggagagtgttga

SEQ ID NO: 127 - DNA, 1353 bp, synthetic construct
  source 1..1353: mol_type = other DNA; note = Antibody z11 Heavy Chain DNA Sequences
caggtgcagctggtgcagagcggagccgaggtgaagaagcctggcgccagcgtgaaggtgagctgcaaggccagcggctacaccttcaccaactacggcatgaactgggtgaggcaggctcctggccagggactggagtggatgggctggatcaacacctacaccggcgagcccacctacgccgacgacttcaagggcagggtgaccatgaccctggacaccagcaccagcaccgcctacatggagctgaggagcctgaggagcgacgacatggccgtgtactactgcgccaggaagagcaccgtggtgtccaggtacttcgacgtgtggggacagggcaccaccgtgaccgtgagcagcgcgtcgaccaagggcccatccgtcttccccctggcaccctcctccaagagcacctctgggggcacagcggccctgggctgcctggtcaaggactacttccccgaaccggtgacggtgtcctggaactcaggcgctctgaccagcggcgtgcacaccttcccggctgtcctacagtcctcaggactctactccctcagcagcgtggtgaccgtgccctccagcagcttgggcacccagacctacatctgcaacgtgaatcacaagcccagcaacaccaaggtggacaagagagttgagcccaaatcttgtgacaaaactcacacatgcccaccgtgcccagcacctgaactcctggggggaccgtcagtcttcctcttccccccaaaacccaaggacaccctcatgatctcccggacccctgaggtcacatgcgtggtggtggacgtgagccacgaagaccctgaggtcaagttcaactggtacgtggacggcgtggaggtgcataatgccaagacaaagccgcgggaggagcagtacaacagcacgtaccgtgtggtcagcgtcctcaccgtcctgcaccaggactggctgaatggcaaggagtacaagtgcaaggtctccaacaaagccctcccagcccccatcgagaaaaccatctccaaagccaaagggcagccccgagaaccacaggtctacaccctgcccccatcccgggaggagatgaccaagaaccaggtcagcctgacctgcctggtcaaaggcttctatcccagcgacatcgccgtggagtgggagagcaatgggcagccggagaacaactacaagaccacgcctcccgtgctggactccgacggctccttcttcctctatagcaagctcaccgtggacaagagcaggtggcagcaggggaacgtcttctcatgctccgtgatgcatgaggctctgcacaaccactacacgcagaagagcttaagcctgtctccgggtaaatga

SEQ ID NO: 128 - DNA, 1353 bp, synthetic construct
  source 1..1353: mol_type = other DNA; note = Antibody z13 Heavy Chain DNA Sequences
caggtgcagctggtgcagagcggagccgaagtgaagaagcccggcgccagcgtgaaggtgagctgcaaggccagcggctacaccttcaccaactacggcatgaactgggtgagacaggcccctggacagggactggagtggatgggctggatcaacacctacaccggcgagcccacctacgccgacgacttcaagggcagggtgaccttcaccctggacaccagcaccagcaccgcctacatggagctgaggagcctgaggagcgacgacatggccgtgtactattgcgccaggaagagcaccgtggtgagcaggtacttcgacgtgtggggccagggaaccaccgtgaccgtgagcagcgcgtcgaccaagggcccatccgtcttccccctggcaccctcctccaagagcacctctgggggcacagcggccctgggctgcctggtcaaggactacttccccgaaccggtgacggtgtcctggaactcaggcgctctgaccagcggcgtgcacaccttcccggctgtcctacagtcctcaggactctactccctcagcagcgtggtgaccgtgccctccagcagcttgggcacccagacctacatctgcaacgtgaatcacaagcccagcaacaccaaggtggacaagagagttgagcccaaatcttgtgacaaaactcacacatgcccaccgtgcccagcacctgaactcctggggggaccgtcagtcttcctcttccccccaaaacccaaggacaccctcatgatctcccggacccctgaggtcacatgcgtggtggtggacgtgagccacgaagaccctgaggtcaagttcaactggtacgtggacggcgtggaggtgcataatgccaagacaaagccgcgggaggagcagtacaacagcacgtaccgtgtggtcagcgtcctcaccgtcctgcaccaggactggctgaatggcaaggagtacaagtgcaaggtctccaacaaagccctcccagcccccatcgagaaaaccatctccaaagccaaagggcagccccgagaaccacaggtctacaccctgcccccatcccgggaggagatgaccaagaaccaggtcagcctgacctgcctggtcaaaggcttctatcccagcgacatcgccgtggagtgggagagcaatgggcagccggagaacaactacaagaccacgcctcccgtgctggactccgacggctccttcttcctctatagcaagctcaccgtggacaagagcaggtggcagcaggggaacgtcttctcatgctccgtgatgcatgaggctctgcacaaccactacacgcagaagagcttaagcctgtctccgggtaaatga

SEQ ID NO: 129 - DNA, 1353 bp, synthetic construct
  source 1..1353: mol_type = other DNA; note = Antibody xAb Heavy Chain DNA Sequences
cagatccagttggtgcagtctggacctgagctgaagaagcctggagagacagtcaagatctcctgcaaggcttctggatataccttcacaaactatggaatgaactgggtgaagcaggctccaggaaagggtttaaagtggatgggctggataaacacctacactggagagccaacatatgctgatgacttcaagggacggtttgtcttctctttggaaacctctgccagcactgcctacttgcagatcaacaacctcaaaaatgaggacatggccacatatttctgtgcaagaaaaagtacggtagtaagtaggtacttcgatgtctggggcgcagggaccacggtcaccgtctcctcagcgtcgaccaagggcccatccgtcttccccctggcaccctcctccaagagcacctctgggggcacagcggccctgggctgcctggtcaaggactacttccccgaaccggtgacggtgtcctggaactcaggcgctctgaccagcggcgtgcacaccttcccggctgtcctacagtcctcaggactctactccctcagcagcgtggtgaccgtgccctccagcagcttgggcacccagacctacatctgcaacgtgaatcacaagcccagcaacaccaaggtggacaagagagttgagcccaaatcttgtgacaaaactcacacatgcccaccgtgcccagcacctgaactcctggggggaccgtcagtcttcctcttccccccaaaacccaaggacaccctcatgatctcccggacccctgaggtcacatgcgtggtggtggacgtgagccacgaagaccctgaggtcaagttcaactggtacgtggacggcgtggaggtgcataatgccaagacaaagccgcgggaggagcagtacaacagcacgtaccgtgtggtcagcgtcctcaccgtcctgcaccaggactggctgaatggcaaggagtacaagtgcaaggtctccaacaaagccctcccagcccccatcgagaaaaccatctccaaagccaaagggcagccccgagaaccacaggtctacaccctgcccccatcccgggaggagatgaccaagaaccaggtcagcctgacctgcctggtcaaaggcttctatcccagcgacatcgccgtggagtgggagagcaatgggcagccggagaacaactacaagaccacgcctcccgtgctggactccgacggctccttcttcctctatagcaagctcaccgtggacaagagcaggtggcagcaggggaacgtcttctcatgctccgtgatgcatgaggctctgcacaaccactacacgcagaagagcttaagcctgtctccgggtaaatga

SEQ ID NO: 130 - DNA, 645 bp, synthetic construct
  source 1..645: mol_type = other DNA; note = Antibody xAb Light Chain DNA Sequences
gacattgtgctgacccagtctcacaaattcatgtccacatcagtaggagacagggtcagcatcacctgcaaggccagtcaggatgtgggtgatgctgtaacctggtgtcaacagaaaccaggtcaacctcctaaactactgatttactgggcatccacccggcacactggagtccctgatcgcttcacaggcagtgggtctgggacagatttcactctcaccattaacaatgtgcagtctgaggacttggcagattatttctgtcagcaatatcgcagctatcctctcacgttcggtgctgggaccaagctggagctgaaacgtacggtggctgcaccatctgtcttcatcttcccgccatctgatgagcagttgaaatctggaactgcctctgttgtgtgcctgctgaataacttctatcccagagaggccaaagtacagtggaaggtggataacgccctccaatcgggtaactcccaggagagtgtcacagagcaggacagcaaggacagcacctacagcctcagcagcaccctgacgctgagcaaagcagactacgagaaacacaaagtctacgcctgcgaagtcacccatcagggcctgagctcgcccgtcacaaagagcttcaacaggggagagtgttga

SEQ ID NO: 131 - protein, 999 aa, Homo sapiens
  source 1..999: note = Full-Length Human MERTK (Swiss-Prot ID: Q12866.2)
MGPAPLPLLLGLFLPALWRRAITEAREEAKPYPLFPGPFPGSLQTDHTPLLSLPHASGYQPALMFSPTQPGRPHTGNVAIPQVTSVESKPLPPLAFKHTVGHIILSEHKGVKFNCSISVPNIYQDTTISWWKDGKELLGAHHAITQFYPDDEVTAIIASFSITSVQRSDNGSYICKMKINNEEIVSDPIYIEVQGLPHFTKQPESMNVTRNTAFNLTCQAVGPPEPVNIFWVQNSSRVNEQPEKSPSVLTVPGLTEMAVFSCEAHNDKGLTVSKGVQINIKAIPSPPTEVSIRNSTAHSILISWVPGFDGYSPFRNCSIQVKEADPLSNGSVMIFNTSALPHLYQIKQLQALANYSIGVSCMNEIGWSAVSPWILASTTEGAPSVAPLNVTVFLNESSDNVDIRWMKPPTKQQDGELVGYRISHVWQSAGISKELLEEVGQNGSRARISVQVHNATCTVRIAAVTRGGVGPFSDPVKIFIPAHGWVDYAPSSTPAPGNADPVLIIFGCFCGFILIGLILYISLAIRKRVQETKFGNAFTEEDSELVVNYIAKKSFCRRAIELTLHSLGVSEELQNKLEDVVIDRNLLILGKILGEGEFGSVMEGNLKQEDGTSLKVAVKTMKLDNSSQREIEEFLSEAACMKDFSHPNVIRLLGVCIEMSSQGIPKPMVILPFMKYGDLHTYLLYSRLETGPKHIPLQTLLKFMVDIALGMEYLSNRNFLHRDLAARNCMLRDDMTVCVADFGLSKKIYSGDYYRQGRIAKMPVKWIAIESLADRVYTSKSDVWAFGVTMWEIATRGMTPYPGVQNHEMYDYLLHGHRLKQPEDCLDELYEIMYSCWRTDPLDRPTFSVLRLQLEKLLESLPDVRNQADVIYVNTQLLESSEGLAQGSTLAPLDLNIDPDSIIASCTPRAAISVVTAEVHDSKPHEGRYILNGGSEEWEDLTSAPSAAVTAEKNSVLPGERLVRNGVSWSHSSMLPLGSSLPDELLFADDSSEGSEVLM

SEQ ID NO: 132 - protein, 474 aa, synthetic construct
  source 1..474: note = Extracellular Domain of MERTK Used for Immunization
REEAKPYPLFPGPFPGSLQTDHTPLLSLPHASGYQPALMFSPTQPGRPHTGNVAIPQVTSVESKPLPPLAFKHTVGHIILSEHKGVKFNCSISVPNIYQDTTISWWKDGKELLGAHHAITQFYPDDEVTAIIASFSITSVQRSDNGSYICKMKINNEEIVSDPIYIEVQGLPHFTKQPESMNVTRNTAFNLTCQAVGPPEPVNIFWVQNSSRVNEQPEKSPSVLTVPGLTEMAVFSCEAHNDKGLTVSKGVQINIKAIPSPPTEVSIRNSTAHSILISWVPGFDGYSPFRNCSIQVKEADPLSNGSVMIFNTSALPHLYQIKQLQALANYSIGVSCMNEIGWSAVSPWILASTTEGAPSVAPLNVTVFLNESSDNVDIRWMKPPTKQQDGELVGYRISHVWQSAGISKELLEEVGQNGSRARISVQVHNATCTVRIAAVTRGGVGPFSDPVKIFIPAHGWVDYAPSSTPAPGNA